European Patent Application EP 4 202 064 A1, published June 28, 2023. Title: KIT AND METHOD FOR ISOTHERMAL RAPID DETECTION OF SARS-COV-2 VIRUS NUCLEIC ACID. Applicant: SHANGHAI JIAO TONG UNIVERSITY. Application EP21857715.3. The sequence listing filed with the application follows.

SEQUENCE LISTING (71 sequences)

SEQ ID NO: 1 - DNA, 19 bp, artificial sequence
  primer
atcagtactagtgcctgtg

SEQ ID NO: 2 - DNA, 18 bp, artificial sequence
  primer
tgttgtctgtactgccgt

SEQ ID NO: 3 - DNA, 40 bp, artificial sequence
  primer
tagttgtgatcaactccgcgaatgcacttacaccgcaaac

SEQ ID NO: 4 - DNA, 46 bp, artificial sequence
  primer
agcacaagttgtaggtatttgtacatgccacatagatcatccaaat

SEQ ID NO: 5 - DNA, 23 bp, artificial sequence
  primer
cagctgatgcacaatcgttttta

SEQ ID NO: 6 - DNA, 25 bp, artificial sequence
  primer
ccttttaagtcacaaaatcctttag

SEQ ID NO: 7 - DNA, 22 bp, artificial sequence
  primer
gaatttagcaaaaccagctact

SEQ ID NO: 8 - DNA, 18 bp, artificial sequence
  primer
gtgttgtctgtactgccg

SEQ ID NO: 9 - DNA, 43 bp, artificial sequence
  primer
cgtttttaaacgggtttgcggtatacgacatcagtactagtgc

SEQ ID NO: 10 - DNA, 46 bp, artificial sequence
  primer
tgtaaaacccacagggtcattagcccaaatcctaaaggattttgtg

SEQ ID NO: 11 - DNA, 18 bp, artificial sequence
  primer
tgcagcccgtcttacacc

SEQ ID NO: 12 - DNA, 25 bp, artificial sequence
  primer
caagttgtaggtatttgtacatact

SEQ ID NO: 13 - DNA, 18 bp, artificial sequence
  primer
tgttcttgctcgcaaaca

SEQ ID NO: 14 - DNA, 20 bp, artificial sequence
  primer
gtgttgtaaattgcggacat

SEQ ID NO: 15 - DNA, 43 bp, artificial sequence
  primer
acacatgaccatttcactcaatactagcttgtcacaccgtttc

SEQ ID NO: 16 - DNA, 43 bp, artificial sequence
  primer
catttgtcaagctgtcacggcgcaattttgttaccatcagtag

SEQ ID NO: 17 - DNA, 17 bp, artificial sequence
  primer
acactcattagctaatc

SEQ ID NO: 18 - DNA, 18 bp, artificial sequence
  primer
caatgttaatgcactttt

SEQ ID NO: 19 - DNA, 20 bp, artificial sequence
  primer
cgcaaacatacaacgtgttg

SEQ ID NO: 20 - DNA, 20 bp, artificial sequence
  primer
gtgttgtaaattgcggacat

SEQ ID NO: 21 - DNA, 43 bp, artificial sequence
  primer
acacatgaccatttcactcaatactgcttgtcacaccgtttct

SEQ ID NO: 22 - DNA, 42 bp, artificial sequence
  primer
catttgtcaagctgtcacggcggcaattttgttaccatcagt

SEQ ID NO: 23 - DNA, 21 bp, artificial sequence
  primer
cacactcattagctaatctat

SEQ ID NO: 24 - DNA, 21 bp, artificial sequence
  primer
caatgttaatgcacttttatc

SEQ ID NO: 25 - DNA, 19 bp, artificial sequence
  primer
tctgccgaaagcttgtgtt

SEQ ID NO: 26 - DNA, 20 bp, artificial sequence
  primer
cgtagtcgcaacagttcaag

SEQ ID NO: 27 - DNA, 42 bp, artificial sequence
  primer
gccaacaacaacaaggccaaactcagtacgtttttgccgagg

SEQ ID NO: 28 - DNA, 39 bp, artificial sequence
  primer
gcatcaccgccattgccagccaactccaggcagcagtag

SEQ ID NO: 29 - DNA, 21 bp, artificial sequence
  primer
gctgctgaggcttctaagaag

SEQ ID NO: 30 - DNA, 21 bp, artificial sequence
  primer
attctagcaggagaagttccc

SEQ ID NO: 31 - DNA, 19 bp, artificial sequence
  primer
tctgccgaaagcttgtgtt

SEQ ID NO: 32 - DNA, 19 bp, artificial sequence
  primer
cagtcaagcctcttctcgt

SEQ ID NO: 33 - DNA, 42 bp, artificial sequence
  primer
ccaacaacaacaaggccaaactggcagtacgtttttgccgag

SEQ ID NO: 34 - DNA, 41 bp, artificial sequence
  primer
accgccattgccagccattctaacgtagtcgcaacagttca

SEQ ID NO: 35 - DNA, 21 bp, artificial sequence
  primer
tgctgctgaggcttctaagaa

SEQ ID NO: 36 - DNA, 21 bp, artificial sequence
  primer
gttcccctactgctgcctgga

SEQ ID NO: 37 - DNA, 17 bp, artificial sequence
  primer
ttgatgagctggagcca

SEQ ID NO: 38 - DNA, 18 bp, artificial sequence
  primer
caccctcaatgcagagtc

SEQ ID NO: 39 - DNA, 41 bp, artificial sequence
  primer
gtgtgaccctgaagactcggttttagccactgactcggatc

SEQ ID NO: 40 - DNA, 45 bp, artificial sequence
  primer
cctccgtgatatggctcttcgtttttttcttacatggctctggtc

SEQ ID NO: 41 - DNA, 20 bp, artificial sequence
  primer
atgtggatggctgagttgtt

SEQ ID NO: 42 - DNA, 20 bp, artificial sequence
  primer
catgctgagtactggacctc

SEQ ID NO: 43 - DNA, 17 bp, artificial sequence
  primer
ggagccagagaccgaca

SEQ ID NO: 44 - DNA, 17 bp, artificial sequence
  primer
ctcaggaaggcccacta

SEQ ID NO: 45 - DNA, 40 bp, artificial sequence
  primer
ttacttgggtgtgaccctgaagacacgggagccactgact

SEQ ID NO: 46 - DNA, 40 bp, artificial sequence
  primer
aagaaaaggcctgttccctggaaggccaccaagagacaat

SEQ ID NO: 47 - DNA, 20 bp, artificial sequence
  primer
tggatggctgagttgttgcg

SEQ ID NO: 48 - DNA, 21 bp, artificial sequence
  primer
gcccaaaggactctgcattga

SEQ ID NO: 49 - DNA, 16 bp, artificial sequence
  the guide ssDNA
tgtatgtggaaaggtt

SEQ ID NO: 50 - DNA, 16 bp, artificial sequence
  the guide ssDNA
tgtctgtaccgtctgc

SEQ ID NO: 51 - DNA, 16 bp, artificial sequence
  the guide ssDNA
ttgatgaggttccacc

SEQ ID NO: 52 - DNA, 16 bp, artificial sequence
  the guide ssDNA
tcagttgtggcatctc

SEQ ID NO: 53 - DNA, 16 bp, artificial sequence
  the guide ssDNA
taggtggaacctcatc

SEQ ID NO: 54 - DNA, 16 bp, artificial sequence
  the guide ssDNA
tggagatgccacaact

SEQ ID NO: 55 - DNA, 16 bp, artificial sequence
  the guide ssDNA
tcttgacagattgaac

SEQ ID NO: 56 - DNA, 16 bp, artificial sequence
  the guide ssDNA
tcttgctttgctgctg

SEQ ID NO: 57 - DNA, 16 bp, artificial sequence
  the guide ssDNA
tactcagcatgcgaag

SEQ ID NO: 58 - DNA, 16 bp, artificial sequence
  the guide ssDNA
tgccatatcacggagg

SEQ ID NO: 59 - DNA, 30 bp, artificial sequence
  the guide ssDNA
agtctgtaccgtctgcggtatgtggaaagg

SEQ ID NO: 60 - DNA, 30 bp, artificial sequence
  the guide ssDNA
cagttgtggcatctcctgatgaggttccac

SEQ ID NO: 61 - DNA, 30 bp, artificial sequence
  the guide ssDNA
gtggaacctcatcaggagatgccacaactg

SEQ ID NO: 62 - DNA, 30 bp, artificial sequence
  the guide ssDNA
ctcttgctttgctgctgcttgacagattga

SEQ ID NO: 63 - DNA, 30 bp, artificial sequence
  the guide ssDNA
ctcagcatgcgaagagccatatcacggagg

SEQ ID NO: 64 - DNA, 30 bp, artificial sequence; identical to SEQ ID NO: 63
  the guide ssDNA

SEQ ID NO: 65 - DNA, 1000 bp, artificial sequence
  the specific target nucleic acid
atgcacttttcgcatatacaaaacgtaatgtcatccctactataactcaaatgaatcttaagtatgccattagtgcaaagaatagagctcgcaccgtagctggtgtctctatctgtagtactatgaccaatagacagtttcatcaaaaattattgaaatcaatagccgccactagaggagctactgtagtaattggaacaagcaaattctatggtggttggcacaacatgttaaaaactgtttatagtgatgtagaaaaccctcaccttatgggttgggattatcctaaatgtgatagagccatgcctaacatgcttagaattatggcctcacttgttcttgctcgcaaacatacaacgtgttgtagcttgtcacaccgtttctatagattagctaatgagtgtgctcaagtattgagtgaaatggtcatgtgtggcggttcactatatgttaaaccaggtggaacctcatcaggagatgccacaactgcttatgctaatagtgtttttaacatttgtcaagctgtcacggccaatgttaatgcacttttatctactgatggtaacaaaattgccgataagtatgtccgcaatttacaacacagactttatgagtgtctctatagaaatagagatgttgacacagactttgtgaatgagttttacgcatatttgcgtaaacatttctcaatgatgatactctctgacgatgctgttgtgtgtttcaatagcacttatgcatctcaaggtctagtggctagcataaagaactttaagtcagttctttattatcaaaacaatgtttttatgtctgaagcaaaatgttggactgagactgaccttactaaaggacctcatgaattttgctctcaacatacaatgctagttaaacagggtgatgattatgtgtaccttccttacccagatccatcaagaatcctaggggccggctgttttgtagatgatatcgtaaaaacagatggtacacttatgattgaacg

SEQ ID NO: 66 - DNA, 30 bp, artificial sequence
  reporter
ctgtgcagttaacgtcctgataaagaacag

SEQ ID NO: 67 - DNA, 30 bp, artificial sequence
  reporter
ctgtgcagttaacctcctgataaagaacag

SEQ ID NO: 68 - DNA, 30 bp, artificial sequence
  reporter
ctgtgcagttaacttcctgataaagaacag

SEQ ID NO: 69 - DNA, 30 bp, artificial sequence
  reporter
ctgtgcagttaactccctgataaagaacag

SEQ ID NO: 70 - DNA, 30 bp, artificial sequence
  reporter
ctgtgcagttaacgccctgataaagaacag

SEQ ID NO: 71 - DNA, 30 bp, artificial sequence
  reporter
ctgtgcagttaaccccctgataaagaacag